European Patent Specification EP 3 233 888 B1, published February 22, 2023. Title: IMMUNOMODULATORS. Applicant: Bristol-Myers Squibb Company. The sequence listing filed with the application follows.

SEQUENCE LISTING (2 sequences)

SEQ ID NO: 1 - protein, 384 aa, Homo sapiens
LDSPDRPWNPPTFSPALLVVTEGDNATFTCSFSNTSESFVLNWYRMSPSNQTDKLAAFPEDRSQPGQDCRFRVTQLPNGRDFHMSVVRARRNDSGTYLCGAISLAPKAQIKESLRAELRVTERRAEVPTAHPSPSPRPAGQFQGSPGGGGGREPKSSDKTHTSPPSPAPELLGGSSVFLFPPKPKDTLMISRTPEVTCVVVDVSHEDPEVKFNWYVDGVEVHNAKTKPREEQYNSTYRVVSVLTVLHQDWLNGKEYKCKVSNKALPAPIEKTISKAKGQPREPQVYTLPPSRDELTKNQVSLTCLVKGFYPSDIAVEWESNGQPENNYKTTPPVLDSDGSFFLYSKLTVDKSRWQQGNVFSCSVMHEALHNHYTQKSLSLSPGK

SEQ ID NO: 2 - protein, 237 aa, Homo sapiens
FTVTVPKDLYVVEYGSNMTIECKFPVEKQLDLAALIVYWEMEDKNIIQFVHGEEDLKVQHSSYRQRARLLKDQLSLGNAALQITDVKLQDAGVYRCMISYGGADYKRITVKVNAPYNKINQRILVVDPVTSEHELTCQAEGYPKAEVIWTSSDHQVLSGKTTTTNSKREEKLFNVTSTLRINTTTNEIFYCTFRRLDPEENHTAELVIPELPLAHPPNERTGSSETVRFQGHHHHHH